European Patent Application EP 4 609 870 A2, published September 3, 2025. Title: FC-EPSILON CAR. Applicant: ImmunityBio, Inc. Application EP. The sequence listing filed with the application follows.

SEQUENCE LISTING (53 sequences)

SEQ ID NO: 1 - protein, 41 aa, synthetic construct
  REGION 1..41: note = FceRIgamma intracellular
LKIQVRKAAITSYEKSDGVYTGLSTRNQETYETLKHEKPPQ

SEQ ID NO: 2 - DNA, 123 bp, synthetic construct
  misc_feature 1..123: note = FceR1gamma for the Intracellular Signaling Domain
  source 1..123: mol_type = other DNA
ctgaagatccaggtccgaaaggccgccatcaccagctacgagaagtctgatggcgtgtacaccggcctgagcaccagaaaccaggaaacctacgagacactgaagcacgagaagcccccccag

SEQ ID NO: 3 - protein, 54 aa, synthetic construct
  REGION 1..54: note = CD8 Hinge
FVPVFLPAKPTTTPAPRPPTPAPTIASQPLSLRPEACRPAAGGAVHTRGLDFAC

SEQ ID NO: 4 - protein, 65 aa, synthetic construct
  REGION 1..65: note = CD8 Hinge
ALSNSIMYFSHFVPVFLPAKPTTTPAPRPPTPAPTIASQPLSLRPEACRPAAGGAVHTRGLDFAC

SEQ ID NO: 5 - DNA, 195 bp, synthetic construct
  misc_feature 1..195: note = CD8a Hinge DNA
  source 1..195: mol_type = other DNA
gcgctgagcaacagcatcatgtacttcagccacttcgtgcctgtgttcctgcctgccaagcctacaacaacaccagcccctagacctccaacccctgcccctacaattgcctctcagcctctgtctctgaggcccgaagcttgtagacctgctgctggcggagctgtgcacaccagaggactggatttcgcctgc

SEQ ID NO: 6 - protein, 28 aa, synthetic construct
  REGION 1..28: note = CD28 Transmembrane
FWVLVVVGGVLACYSLLVTVAFIIFWVR

SEQ ID NO: 7 - DNA, 84 bp, synthetic construct
  misc_feature 1..84: note = CD28 for the Transmembrane DNA
  source 1..84: mol_type = other DNA
ttttgggtgctggtggtcgtgggcggagtgctggcttgttattctctgctggtcaccgtggccttcatcatcttttgggtccga

SEQ ID NO: 8 - protein, 134 aa, synthetic construct
  REGION 1..134: note = CD8 hinge region, CD28 transmembrane, and FceRIgamma signaling domain
ALSNSIMYFSHFVPVFLPAKPTTTPAPRPPTPAPTIASQPLSLRPEACRPAAGGAVHTRGLDFACFWVLVVVGGVLACYSLLVTVAFIIFWVRLKIQVRKAAITSYEKSDGVYTGLSTRNQETYETLKHEKPPQ

SEQ ID NO: 9 - DNA, 402 bp, synthetic construct
  misc_feature 1..402: note = CD8 hinge, CD28 transmembrane, and FceRIgamma signaling domain DNA
  source 1..402: mol_type = other DNA
gcgctgagcaacagcatcatgtacttcagccacttcgtgcctgtgttcctgcctgccaagcctacaacaacaccagcccctagacctccaacccctgcccctacaattgcctctcagcctctgtctctgaggcccgaagcttgtagacctgctgctggcggagctgtgcacaccagaggactggatttcgcctgcttttgggtgctggtggtcgtgggcggagtgctggcttgttattctctgctggtcaccgtggccttcatcatcttttgggtccgactgaagatccaggtccgaaaggccgccatcaccagctacgagaagtctgatggcgtgtacaccggcctgagcaccagaaaccaggaaacctacgagacactgaagcacgagaagcccccccag

SEQ ID NO: 10 - protein, 398 aa, synthetic construct
  REGION 1..398: note = CD19CAR_ FceRIgamma
MDWIWRILFLVGAATGAHSAQPADIQMTQTTSSLSASLGDRVTISCRASQDISKYLNWYQQKPDGTVKLLIYHTSRLHSGVPSRFSGSGSGTDYSLTISNLEQEDIATYFCQQGNTLPYTFGGGTKLELKRGGGGSGGGGSGGGGSGGGGSEVQLQQSGPGLVAPSQSLSVTCTVSGVSLPDYGVSWIRQPPRKGLEWLGVIWGSETTYYNSALKSRLTIIKDNSKSQVFLKMNSLQTDDTAIYYCAKHYYYGGSYAMDYWGQGTTVTVSSAAALFVPVFLPAKPTTTPAPRPPTPAPTIASQPLSLRPEACRPAAGGAVHTRGLDFACFWVLVVVGGVLACYSLLVTVAFIIFWVRLKIQVRKAAITSYEKSDGVYTGLSTRNQETYETLKHEKPPQ

SEQ ID NO: 11 - protein, 255 aa, synthetic construct
  REGION 1..255: note = Anti-CD19 scFv
AQPADIQMTQTTSSLSASLGDRVTISCRASQDISKYLNWYQQKPDGTVKLLIYHTSRLHSGVPSRFSGSGSGTDYSLTISNLEQEDIATYFCQQGNTLPYTFGGGTKLELKRGGGGSGGGGSGGGGSGGGGSEVQLQQSGPGLVAPSQSLSVTCTVSGVSLPDYGVSWIRQPPRKGLEWLGVIWGSETTYYNSALKSRLTIIKDNSKSQVFLKMNSLQTDDTAIYYCAKHYYYGGSYAMDYWGQGTTVTVSSAAA

SEQ ID NO: 12 - DNA, 1197 bp, synthetic construct
  misc_feature 1..1197: note = CD19CAR_ FceRIgamma DNA
  source 1..1197: mol_type = other DNA
atggactggatctggcggattctgtttctcgtgggagctgccacaggcgctcattctgctcagcctgccgatatccagatgacccagacaacaagcagcctgagcgcctctctgggcgatagagtgacaatcagctgcagagccagccaggacatcagcaagtacctgaactggtatcagcagaaacccgacggcaccgtgaagctgctgatctaccacacaagcagactgcacagcggcgtgccaagcagattttctggcagcggcagcggcaccgattacagcctgaccatcagcaacctggaacaggaagatatcgctacctacttctgtcagcagggcaacaccctgccttacacctttggcggcggaacaaagctggaactgaaaagaggcggcggaggaagcggaggcggaggatctgggggcggaggctctggcggagggggatctgaagtgcagctgcagcagtctggacctggactggtggctccttctcagtccctgtctgtgacctgtacagtgtctggcgtgtccctgcctgattacggcgtgtcctggatcagacagcctcccagaaaaggcctggaatggctgggagtgatctggggcagcgagacaacctactacaacagcgccctgaagtcccggctgaccatcatcaaggacaacagcaagagccaggtgttcctgaagatgaacagcctgcagaccgacgacaccgccatctactactgcgccaagcactactactacggcggcagctacgccatggattattggggccagggcaccaccgtgacagtgtcatctgctgctgctctgttcgtgcctgtgttcctgcctgccaagcctacaacaacaccagcccctagacctccaacccctgcccctacaattgcctctcagcctctgtctctgaggcccgaagcttgtagacctgctgctggcggagctgtgcacaccagaggactggatttcgcctgcttttgggtgctggtggtcgtgggcggagtgctggcttgttattctctgctggtcaccgtggccttcatcatcttttgggtccgactgaagatccaggtccgaaaggccgccatcaccagctacgagaagtctgatggcgtgtacaccggcctgagcaccagaaaccaggaaacctacgagacactgaagcacgagaagcccccccagtaa

SEQ ID NO: 13 - protein, 41 aa, synthetic construct
  REGION 1..41: note = CD28 signaling domain
RSKRSRLLHSDYMNMTPRRPGPTRKHYQPYAPPRDFAAYRS

SEQ ID NO: 14 - protein, 42 aa, synthetic construct
  REGION 1..42: note = 4-1BB signaling domain
KRGRKKLLYIFKQPFMRPVQTTQEEDGCSCRFPEEEEGGCEL

SEQ ID NO: 15 - protein, 113 aa, synthetic construct
  REGION 1..113: note = CD3 zeta signaling domain
RVKFSRSADAPAYQQGQNQLYNELNLGRREEYDVLDKRRGRDPEMGGKPQRRKNPQEGLYNELQKDKMAEAYSEIGMKGERRRGKGHDGLYQGLSTATKDTYDALHMQALPPR

SEQ ID NO: 16 - DNA, 1410 bp, synthetic construct
  misc_feature 1..1410: note = CD19CAR_CD3z
  source 1..1410: mol_type = other DNA
atggactggatctggcggatcctgtttctcgtgggagctgccacaggcgctcattctgctcagcctgccgatatccagatgacccagacaacaagcagcctgagcgcctctctgggcgatagagtgacaatcagctgcagagccagccaggacatcagcaagtacctgaactggtatcagcagaaacccgacggcaccgtgaagctgctgatctaccacacaagcagactgcacagcggcgtgccaagcagattttctggcagcggcagcggcaccgattacagcctgaccatcagcaacctggaacaggaagatatcgctacctacttctgtcagcaaggcaacaccctgccttacacctttggcggcggaacaaagctggaactgaaaagaggcggcggaggaagcggaggcggaggatctgggggcggaggctctggcggagggggatctgaagtgcagctgcagcagtctggacctggactggtggctccttctcagtccctgtctgtgacctgtacagtgtctggcgtgtccctgcctgattacggcgtgtcctggatcagacagcctcccagaaaaggcctggaatggctgggagtgatctggggcagcgagacaacctactacaacagcgccctgaagtcccggctgaccatcatcaaggacaacagcaagagccaggtgttcctgaagatgaacagcctgcagaccgacgacaccgccatctactactgcgccaagcactactactacggcggcagctacgccatggattattggggccagggcaccaccgtgacagtgtcatctgctgctgctctgttcgtgcctgtgttcctgcctgccaagcctacaacaacaccagcccctagacctccaacccctgcccctacaattgcctctcagcctctgtctctgaggcccgaagcttgtagacctgctgctggcggagctgtgcacaccagaggactggatttcgcctgcttttgggtgctggtggtcgtgggcggagtgctggcttgttattctctgctggtcaccgtggccttcatcatcttttgggtccgagtgaagttcagcagatccgccgatgcccctgcttaccagcagggccagaatcagctgtacaacgagctgaacctgggcagacgggaagagtacgacgtgctggataagagaagaggcagagatcccgagatgggcggcaagccccagagaagaaagaatccccaggaaggcctgtataacgaactgcagaaagacaagatggccgaggcctacagcgagatcggcatgaagggcgagagaagaagaggcaagggccacgatggactgtaccagggactgagcacagccaccaaggatacctacgatgccctgcacatgcaggccctgcctccaagataa

SEQ ID NO: 17 - DNA, 1533 bp, synthetic construct
  misc_feature 1..1533: note = CD19CAR_CD28/CD3z
  source 1..1533: mol_type = other DNA
atggactggatctggcggatcctgtttctcgtgggagctgccacaggcgctcattctgctcagcctgccgatatccagatgacccagacaacaagcagcctgagcgcctctctgggcgatagagtgacaatcagctgcagagccagccaggacatcagcaagtacctgaactggtatcagcagaaacccgacggcaccgtgaagctgctgatctaccacacaagcagactgcacagcggcgtgccaagcagattttctggcagcggcagcggcaccgattacagcctgaccatcagcaacctggaacaggaagatatcgctacctacttctgtcagcagggcaacaccctgccttacacctttggcggcggaacaaagctggaactgaaaagaggcggcggaggaagcggaggcggaggatctgggggcggaggctctggcggagggggatctgaagtgcagctgcagcagtctggacctggactggtggctccttctcagtccctgtctgtgacctgtacagtgtctggcgtgtccctgcctgattacggcgtgtcctggatcagacagcctcccagaaaaggcctggaatggctgggagtgatctggggcagcgagacaacctactacaacagcgccctgaagtcccggctgaccatcatcaaggacaacagcaagagccaggtgttcctgaagatgaacagcctgcagaccgacgacaccgccatctactactgcgccaagcactactactacggcggcagctacgccatggattattggggccagggcaccaccgtgacagtgtcatctgctgctgctctgttcgtgcctgtgttcctgcctgccaagcctacaacaacaccagcccctagacctccaacccctgcccctacaattgcctctcagcctctgtctctgaggcccgaagcttgtagacctgctgctggcggagctgtgcacaccagaggactggatttcgcctgcttttgggtgctggtggtcgtgggcggagtgctggcttgttattctctgctggtcaccgtggccttcatcatcttttgggtccgaagcaagcggagcaggctgctgcacagcgactacatgaacatgacccctagaaggcctggccccaccagaaagcactatcagccttacgcccctcccagagacttcgccgcctacagatccagagtgaagttcagcagatctgccgacgcccctgcttaccagcagggccagaatcagctgtacaacgagctgaacctgggcagacgggaagagtacgacgtgctggataagagaagaggcagagatcccgagatgggcggcaagccccagagaagaaagaatccccaggaaggcctgtataacgaactgcagaaagacaagatggccgaggcctacagcgagatcggcatgaagggcgagagaagaagaggcaagggccacgatggactgtaccagggactgagcacagccaccaaggatacctacgatgccctgcacatgcaggccctgcctccaagataa

SEQ ID NO: 18 - DNA, 1536 bp, synthetic construct
  misc_feature 1..1536: note = CD19CAR_4-1BB/CD3z
  source 1..1536: mol_type = other DNA
atggactggatctggcggatcctgtttctcgtgggagctgccacaggcgctcattctgctcagcctgccgatatccagatgacccagacaacaagcagcctgagcgcctctctgggcgatagagtgacaatcagctgcagagccagccaggacatcagcaagtacctgaactggtatcagcagaaacccgacggcaccgtgaagctgctgatctaccacacaagcagactgcacagcggcgtgccaagcagattttctggcagcggcagcggcaccgattacagcctgaccatcagcaacctggaacaggaagatatcgctacctacttctgtcagcagggcaacaccctgccttacacctttggcggcggaacaaagctggaactgaaaagaggcggcggaggaagcggaggcggaggatctgggggcggaggctctggcggagggggatctgaagtgcagctgcagcagtctggacctggactggtggctccttctcagtccctgtctgtgacctgtacagtgtctggcgtgtccctgcctgattacggcgtgtcctggatcagacagcctcccagaaaaggcctggaatggctgggagtgatctggggcagcgagacaacctactacaacagcgccctgaagtcccggctgaccatcatcaaggacaacagcaagagccaggtgttcctgaagatgaacagcctgcagaccgacgacaccgccatctactactgcgccaagcactactactacggcggcagctacgccatggattattggggccagggcaccaccgtgacagtgtcatctgctgctgctctgttcgtgcctgtgttcctgcctgccaagcctacaacaacaccagcccctagacctccaacccctgcccctacaattgcctctcagcctctgtctctgaggcccgaagcttgtagacctgctgctggcggagctgtgcacaccagaggactggatttcgcctgcttttgggtgctggtggtcgtgggcggagtgctggcttgttattctctgctggtcaccgtggccttcatcatcttttgggtcaagcggggcagaaagaagctgctgtacatcttcaagcagcccttcatgaggcccgtgcagaccacacaggaagaggacggctgcagctgtagattccctgaggaagaagaaggcggctgcgagctgagagtgaagtttagcagatctgccgacgcccctgcctaccagcagggacagaatcagctgtacaacgagctgaacctgggcagacgggaagagtacgacgtgctggataagagaagaggcagagatcccgagatgggcggcaagccccagagaagaaagaatccccaggaaggcctgtataacgaactgcagaaagacaagatggccgaggcctacagcgagatcggcatgaagggcgagagaagaagaggcaagggccacgatggactgtaccagggactgagcacagccaccaaggatacctacgatgccctgcacatgcaggccctgcctccaagataa

SEQ ID NO: 19 - DNA, 1659 bp, synthetic construct
  misc_feature 1..1659: note = CD19CAR_CD28/4-1BB/CD3z
  source 1..1659: mol_type = other DNA
atggactggatctggcggatcctgtttctcgtgggagctgccacaggcgctcattctgctcagcctgccgatatccagatgacccagacaacaagcagcctgagcgcctctctgggcgatagagtgacaatcagctgcagagccagccaggacatcagcaagtacctgaactggtatcagcagaaacccgacggcaccgtgaagctgctgatctaccacacaagcagactgcacagcggcgtgccaagcagattttctggcagcggcagcggcaccgattacagcctgaccatcagcaacctggaacaggaagatatcgctacctacttctgtcagcagggcaacaccctgccttacacctttggcggcggaacaaagctggaactgaaaagaggcggcggaggaagcggaggcggaggatctgggggcggaggctctggcggagggggatctgaagtgcagctgcagcagtctggacctggactggtggctccttctcagtccctgtctgtgacctgtacagtgtctggcgtgtccctgcctgattacggcgtgtcctggatcagacagcctcccagaaaaggcctggaatggctgggagtgatctggggcagcgagacaacctactacaacagcgccctgaagtcccggctgaccatcatcaaggacaacagcaagagccaggtgttcctgaagatgaacagcctgcagaccgacgacaccgccatctactactgcgccaagcactactactacggcggcagctacgccatggattattggggccagggcaccaccgtgacagtgtcatctgctgctgctctgttcgtgcctgtgttcctgcctgccaagcctacaacaacaccagcccctagacctccaacccctgcccctacaattgcctctcagcctctgtctctgaggcccgaagcttgtagacctgctgctggcggagctgtgcacaccagaggactggatttcgcctgcttttgggtgctggtggtcgtgggcggagtgctggcttgttattctctgctggtcaccgtggccttcatcatcttttgggtccgaagcaagcggagcaggctgctgcacagcgactacatgaacatgacccctagaaggcctggccccaccagaaagcactatcagccttacgcccctcccagagacttcgccgcctatagatccaagcggggcagaaagaagctgctgtacatcttcaagcagcccttcatgaggcccgtgcagaccacacaggaagaggacggctgcagctgtagattccctgaggaagaagaaggcggctgcgagctgagagtgaagtttagcagatctgccgacgcccctgcctaccagcagggacagaatcagctgtacaacgagctgaacctgggcagacgggaagagtacgacgtgctggataagagaagaggcagagatcccgagatgggcggcaagccccagagaagaaagaatccccaggaaggcctgtataacgaactgcagaaagacaagatggccgaggcctacagcgagatcggcatgaagggcgagagaagaagaggcaagggccacgatggactgtaccagggactgagcacagccaccaaggatacctacgatgccctgcacatgcaggccctgcctccaagataa

SEQ ID NO: 20 - DNA, 1659 bp, synthetic construct
  misc_feature 1..1659: note = CD19CAR_4-1BB/CD3z/CD28
  source 1..1659: mol_type = other DNA
atggactggatctggcggatcctgtttctcgtgggagctgccacaggcgctcattctgctcagcctgccgatatccagatgacccagacaacaagcagcctgagcgcctctctgggcgatagagtgacaatcagctgcagagccagccaggacatcagcaagtacctgaactggtatcagcagaaacccgacggcaccgtgaagctgctgatctaccacacaagcagactgcacagcggcgtgccaagcagattttctggcagcggcagcggcaccgattacagcctgaccatcagcaacctggaacaggaagatatcgctacctacttctgtcagcagggcaacaccctgccttacacctttggcggcggaacaaagctggaactgaaaagaggcggcggaggaagcggaggcggaggatctgggggcggaggctctggcggagggggatctgaagtgcagctgcagcagtctggacctggactggtggctccttctcagtccctgtctgtgacctgtacagtgtctggcgtgtccctgcctgattacggcgtgtcctggatcagacagcctcccagaaaaggcctggaatggctgggagtgatctggggcagcgagacaacctactacaacagcgccctgaagtcccggctgaccatcatcaaggacaacagcaagagccaggtgttcctgaagatgaacagcctgcagaccgacgacaccgccatctactactgcgccaagcactactactacggcggcagctacgccatggattattggggccagggcaccaccgtgacagtgtcatctgctgctgctctgttcgtgcctgtgttcctgcctgccaagcctacaacaacaccagcccctagacctccaacccctgcccctacaattgcctctcagcctctgtctctgaggcccgaagcttgtagacctgctgctggcggagctgtgcacaccagaggactggatttcgcctgcttttgggtgctggtggtcgtgggcggagtgctggcttgttattctctgctggtcaccgtggccttcatcatcttttgggtcaagcggggcagaaagaagctgctgtacatcttcaagcagcccttcatgaggcccgtgcagaccacacaggaagaggacggctgcagctgtagattccctgaggaagaagaaggcggctgcgagctgagagtgaagtttagcagatctgccgacgcccctgcctaccagcagggacagaatcagctgtacaacgagctgaacctgggcagacgggaagagtacgacgtgctggataagagaagaggcagagatcccgagatgggcggcaagccccagagaagaaagaatccccaggaaggcctgtataacgaactgcagaaagacaagatggccgaggcctacagcgagatcggcatgaagggcgagagaagaagaggcaagggccacgatggactgtaccagggactgagcacagccaccaaggatacctacgatgccctgcacatgcaggccctgcctccaagaagaagcaagagatctagactgctgcacagcgactacatgaacatgacccctagaaggcctggccccaccagaaagcactatcagccttacgcccctcccagagacttcgccgcctacagatcttga

SEQ ID NO: 21 - protein, 153 aa, synthetic construct
  REGION 1..153: note = Wild-Type IL-2
MYRMQLLSCIALSLALVTNSAPTSSSTKKTQLQLEHLLLDLQMILNGINNYKNPKLTRMLTFKFYMPKKATELKHLQCLEEELKPLEEVLNLAQSKNFHLRPRDLISNINVIVLELKGSETTFMCEYADETATIVEFLNRWITFCQSIISTLT

SEQ ID NO: 22 - protein, 160 aa, synthetic construct
  REGION 1..160: note = IL-2-ER
MYRMQLLSCIALSLALVTNSAPTSSSTKKTQLQLEHLLLDLQMILNGINNYKNPKLTRMLTFKFYMPKKATELKHLQCLEEELKPLEEVLNLAQSKNFHLRPRDLISNINVIVLELKGSETTFMCEYADETATIVEFLNRWITFCQSIISTLTGSEKDEL

SEQ ID NO: 23 - protein, 220 aa, synthetic construct
  REGION 1..220: note = NP_006130.1 CD28 Human
MLRLLLALNLFPSIQVTGNKILVKQSPMLVAYDNAVNLSCKYSYNLFSREFRASLHKGLDSAVEVCVVYGNYSQQLQVYSKTGFNCDGKLGNESVTFYLQNLYVNQTDIYFCKIEVMYPPPYLDNEKSNGTIIHVKGKHLCPSPLFPGPSKPFWVLVVVGGVLACYSLLVTVAFIIFWVRSKRSRLLHSDYMNMTPRRPGPTRKHYQPYAPPRDFAAYRS

SEQ ID NO: 24 - protein, 135 aa, synthetic construct
  REGION 1..135: note = CD19K_ Transmembrane and Signaling domain
AAVLELLSNSIMYFSHFVPVFLPAKPTTTPAPRPPTPAPTIASQPLSLRPEACRPAAGGAVHTRGLDLLDPKLCYLLDGILFIYGVILTALFLRLKIQVRKAAITSYEKSDGVYTGLSTRNQETYETLKHEKPPQ

SEQ ID NO: 25 - protein, 398 aa, synthetic construct; identical to SEQ ID NO: 10
  REGION 1..398: note = CD19CAR FceRIgamma protein

SEQ ID NO: 26 - DNA, 441 bp, synthetic construct
  misc_feature 1..441: note = 15AD23HC_1805843_CD19K_Eps (879 - 1319)
  source 1..441: mol_type = other DNA
tggggccaagggaccacggtcaccgtctcctcggccgcggttctagagctcttgagcaactccatcatgtacttcagccacttcgtgccggtcttcctgccagcgaagcccaccacgacgccagcgccgcgaccaccaacaccggcgcccaccatcgcgtcgcagcccctgtccctgcgcccagaggcgtgccggccagcggcggggggcgcagtgcacacgagggggctggacctgctggatcccaaactctgctacctgctggatggaatcctcttcatctatggtgtcattctcactgccttgttcctgagactgaagatccaagtgcgaaaggcagctataaccagctatgagaaatcagatggtgtttacacgggcctgagcaccaggaaccaggagacttacgagactctgaagcatgagaaaccaccacagtaa

SEQ ID NO: 27 - DNA, 4278 bp, synthetic construct
  misc_feature 1..4278: note = 15AD23HC_1805843_CD19K_Eps
  source 1..4278: mol_type = other DNA
taatacgactcactatagggagacaagcttgcttgttctttttgcagaagctcagaataaacgctcaactttggcagatcggtaccgaattcgccaccatggactggatctggcgcatcctcttcctcgtcggcgctgctaccggcgctcattcggcccagccggccgacatccagatgacacagactacatcctccctgtctgcctctctgggagacagagtcaccatcagttgcagggcaagtcaggacattagtaaatatttaaattggtatcagcaaaaaccagatggaactgttaaactcctgatctaccatacatcaagattacactcaggagtcccatcaaggttcagtggcagtgggtctggaacagattattctctcaccattagcaacctggagcaagaagatattgccacttacttttgccaacagggtaatacgcttccgtacacgttcggaggggggaccaagctggagctgaaacgtggtggtggtggttctggtggtggtggttctggcggcggcggctccggtggtggtggatccgaggtgcagctgcagcagtctggacctggcctggtggcgccctcacagagcctgtccgtcacatgcactgtctcaggggtctcattacccgactatggtgtaagctggattcgccagcctccacgaaagggtctggagtggctgggagtaatatggggtagtgaaaccacatactataattcagctctcaaatccagactgaccatcatcaaggacaactccaagagccaagttttcttaaaaatgaacagtctgcaaactgatgacacagccatttactactgtgccaaacattattactacggtggtagctatgctatggactactggggccaagggaccacggtcaccgtctcctcggccgcggttctagagctcttgagcaactccatcatgtacttcagccacttcgtgccggtcttcctgccagcgaagcccaccacgacgccagcgccgcgaccaccaacaccggcgcccaccatcgcgtcgcagcccctgtccctgcgcccagaggcgtgccggccagcggcggggggcgcagtgcacacgagggggctggacctgctggatcccaaactctgctacctgctggatggaatcctcttcatctatggtgtcattctcactgccttgttcctgagactgaagatccaagtgcgaaaggcagctataaccagctatgagaaatcagatggtgtttacacgggcctgagcaccaggaaccaggagacttacgagactctgaagcatgagaaaccaccacagtaacagccagggcatttctccctcgagagatctgatatcactagtgactgactaggatctggttaccactaaaccagcctcaagaacacccgaatggagtctctaagctacataataccaacttacactttacaaaatgttgtcccccaaaatgtagccattcgtatctgctcctaataaaaagaaagtttcttcacattctaaaaaaaaaaaaaaaaaaaaaaaaaaaaaaaaacccccccccccccccccctgcaggtcgactctagaggatccccgggtaccgagctcgaattagtattctatagtgtcacctaaatccaattcactggccgtcgttttacaacgtcgtgactgggaaaaccctggcgttacccaacttaatcgccttgcagcacatccccctttcgccagctggcgtaatagcgaagaggcccgcaccgatcgcccttcccaacagttgcgcagcctgaatggcgaatggcgcctgatgcggtattttctccttacgcatctgtgcggtatttcacaccgcatatggtgcactctcagtacaatctgctctgatgccgcatagttaagccagccccgacacccgccaacacccgctgacgcgccctgacgggcttgtctgctcccggcatccgcttacagacaagctgtgaccgtctccgggagctgcatgtgtcagaggttttcaccgtcatcaccgaaacgcgcgagacgaaagggcctcgtgatacgcctatttttataggttaatgtcatgataataatggtttcttagacgtcaggtggcacttttcggggaaatgtgcgcggaacccctatttgtttatttttctaaatacattcaaatatgtatccgctcatgagacaataaccctgataaatgcttcaataatattgaaaaaggaagagtatgagtattcaacatttccgtgtcgcccttattcccttttttgcggcattttgccttcctgtttttgctcacccagaaacgctggtgaaagtaaaagatgctgaagatcagttgggtgcacgagtgggttacatcgaactggatctcaacagcggtaagatccttgagagttttcgccccgaagaacgttttccaatgatgagcacttttaaagttctgctatgtggcgcggtattatcccgtattgacgccgggcaagagcaactcggtcgccgcatacactattctcagaatgacttggttgagtactcaccagtcacagaaaagcatcttacggatggcatgacagtaagagaattatgcagtgctgccataaccatgagtgataacactgcggccaacttacttctgacaacgatcggaggaccgaaggagctaaccgcttttttgcacaacatgggggatcatgtaactcgccttgatcgttgggaaccggagctgaatgaagccataccaaacgacgagcgtgacaccacgatgcctgtagcaatggcaacaacgttgcgcaaactattaactggcgaactacttactctagcttcccggcaacaattaatagactggatggaggcggataaagttgcaggaccacttctgcgctcggcccttccggctggctggtttattgctgataaatctggagccggtgagcgtgggtctcgcggtatcattgcagcactggggccagatggtaagccctcccgtatcgtagttatctacacgacggggagtcaggcaactatggatgaacgaaatagacagatcgctgagataggtgcctcactgattaagcattggtaactgtcagaccaagtttactcatatatactttagattgatttaaaacttcatttttaatttaaaaggatctaggtgaagatcctttttgataatctcatgaccaaaatcccttaacgtgagttttcgttccactgagcgtcagaccccgtagaaaagatcaaaggatcttcttgagatcctttttttctgcgcgtaatctgctgcttgcaaacaaaaaaaccaccgctaccagcggtggtttgtttgccggatcaagagctaccaactctttttccgaaggtaactggcttcagcagagcgcagataccaaatactgttcttctagtgtagccgtagttaggccaccacttcaagaactctgtagcaccgcctacatacctcgctctgctaatcctgttaccagtggctgctgccagtggcgataagtcgtgtcttaccgggttggactcaagacgatagttaccggataaggcgcagcggtcgggctgaacggggggttcgtgcacacagcccagcttggagcgaacgacctacaccgaactgagatacctacagcgtgagctatgagaaagcgccacgcttcccgaagggagaaaggcggacaggtatccggtaagcggcagggtcggaacaggagagcgcacgagggagcttccagggggaaacgcctggtatctttatagtcctgtcgggtttcgccacctctgacttgagcgtcgatttttgtgatgctcgtcaggggggcggagcctatggaaaaacgccagcaacgcggcctttttacggttcctggccttttgctggccttttgctcacatgttctttcctgcgttatcccctgattctgtggataaccgtattaccgcctttgagtgagctgataccgctcgccgcagccgaacgaccgagcgcagcgagtcagtgagcgaggaagcggaagagcgcccaatacgcaaaccgcctctccccgcgcgttggccgattcattaatgcagctggcacgacaggtttcccgactggaaagcgggcagtgagcgcaacgcaattaatgtgagttagctcactcattaggcaccccaggctttacactttatgcttccggctcgtatgttgtgtggaattgtgagcggataacaatttcacacaggaaacagctatgaccatgattacgccaagctc

SEQ ID NO: 28 - DNA, 3136 bp, synthetic construct
  misc_feature 1..3136: note = pNEUKv1_CD19CAR_CD16(158V)_ERIL-2 vector
  source 1..3136: mol_type = other DNA
atggactggatctggcggattctgtttctcgtgggagctgccacaggcgctcattctgctcagcctgccgatatccagatgacccagacaacaagcagcctgagcgcctctctgggcgatagagtgacaatcagctgcagagccagccaggacatcagcaagtacctgaactggtatcagcagaaacccgacggcaccgtgaagctgctgatctaccacacaagcagactgcacagcggcgtgccaagcagattttctggcagcggcagcggcaccgattacagcctgaccatcagcaacctggaacaggaagatatcgctacctacttctgtcagcagggcaacaccctgccttacacctttggcggcggaacaaagctggaactgaaaagaggcggcggaggaagcggaggcggaggatctgggggcggaggctctggcggagggggatctgaagtgcagctgcagcagtctggacctggactggtggctccttctcagtccctgtctgtgacctgtacagtgtctggcgtgtccctgcctgattacggcgtgtcctggatcagacagcctcccagaaaaggcctggaatggctgggagtgatctggggcagcgagacaacctactacaacagcgccctgaagtcccggctgaccatcatcaaggacaacagcaagagccaggtgttcctgaagatgaacagcctgcagaccgacgacaccgccatctactactgcgccaagcactactactacggcggcagctacgccatggattattggggccagggcaccaccgtgacagtgtcatctgcggccgcgctgagcaacagcatcatgtacttcagccacttcgtgcctgtgttcctgcctgccaagcctacaacaacaccagcccctagacctccaacccctgcccctacaattgcctctcagcctctgtctctgaggcccgaagcttgtagacctgctgctggcggagctgtgcacaccagaggactggatttcgcctgcttttgggtgctggtggtcgtgggcggagtgctggcttgttattctctgctggtcaccgtggccttcatcatcttttgggtccgactgaagatccaggtccgaaaggccgccatcaccagctacgagaagtctgatggcgtgtacaccggcctgagcaccagaaaccaggaaacctacgagacactgaagcacgagaagcccccccagggatctggagctactaacttcagcctgctgaagcaggctggagacgtggaggagaaccctggacctatgtggcagctgctgctgcctacagctctcctgctgctggtgtccgccggcatgagaaccgaggatctgcctaaggccgtggtgttcctggaaccccagtggtacagagtgctggaaaaggacagcgtgaccctgaagtgccagggcgcctacagccccgaggacaatagcacccagtggttccacaacgagagcctgatcagcagccaggccagcagctacttcatcgacgccgccaccgtggacgacagcggcgagtatagatgccagaccaacctgagcaccctgagcgaccccgtgcagctggaagtgcacatcggatggctgctgctgcaggcccccagatgggtgttcaaagaagaggaccccatccacctgagatgccactcttggaagaacaccgccctgcacaaagtgacctacctgcagaacggcaagggcagaaagtacttccaccacaacagcgacttctacatccccaaggccaccctgaaggactccggctcctacttctgcagaggcctcgtgggcagcaagaacgtgtccagcgagacagtgaacatcaccatcacccagggcctggccgtgtctaccatcagcagctttttcccacccggctaccaggtgtccttctgcctcgtgatggtgctgctgttcgccgtggacaccggcctgtacttcagcgtgaaaacaaacatcagaagcagcacccgggactggaaggaccacaagttcaagtggcggaaggacccccaggacaagtgaaattccgcccctctcccccccccccctctccctcccccccccctaacgttactggccgaagccgcttggaataaggccggtgtgcgtttgtctatatgttattttccaccatattgccgtcttttggcaatgtgagggcccggaaacctggccctgtcttcttgacgagcattcctaggggtctttcccctctcgccaaaggaatgcaaggtctgttgaatgtcgtgaaggaagcagttcctctggaagcttcttgaagacaaacaacgtctgtagcgaccctttgcaggcagcggaaccccccacctggcgacaggtgcctctgcggccaaaagccacgtgtataagatacacctgcaaaggcggcacaaccccagtgccacgttgtgagttggatagttgtggaaagagtcaaatggctctcctcaagcgtattcaacaaggggctgaaggatgcccagaaggtaccccattgtatgggatctgatctggggcctcggtgcacatgctttacatgtgtttagtcgaggttaaaaaaacgtctaggccccccgaaccacggggacgtggttttcctttgaaaaacacgataaccgccaccatgtaccggatgcagctgctgagctgtatcgccctgtctctggccctcgtgaccaacagcgcccctaccagcagcagcaccaagaaaacccagctgcagctggaacatctgctgctggacctgcagatgatcctgaacggcatcaacaactacaagaaccccaagctgacccggatgctgaccttcaagttctacatgcccaagaaggccaccgaactgaaacatctgcagtgcctggaagaggaactgaagcccctggaagaagtgctgaacctggcccagagcaagaacttccacctgaggcccagggacctgatcagcaacatcaacgtgatcgtgctggaactgaaaggcagcgagacaaccttcatgtgcgagtacgccgacgagacagctaccatcgtggaatttctgaaccggtggatcaccttctgccagagcatcatcagcaccctgaccggctccgagaaggacgagctgtga

SEQ ID NO: 29 - protein, 683 aa, synthetic construct
  REGION 1..683: note = CD19CAR_P2A_CD16(158V) protein
MDWIWRILFLVGAATGAHSAQPADIQMTQTTSSLSASLGDRVTISCRASQDISKYLNWYQQKPDGTVKLLIYHTSRLHSGVPSRFSGSGSGTDYSLTISNLEQEDIATYFCQQGNTLPYTFGGGTKLELKRGGGGSGGGGSGGGGSGGGGSEVQLQQSGPGLVAPSQSLSVTCTVSGVSLPDYGVSWIRQPPRKGLEWLGVIWGSETTYYNSALKSRLTIIKDNSKSQVFLKMNSLQTDDTAIYYCAKHYYYGGSYAMDYWGQGTTVTVSSAAALSNSIMYFSHFVPVFLPAKPTTTPAPRPPTPAPTIASQPLSLRPEACRPAAGGAVHTRGLDFACFWVLVVVGGVLACYSLLVTVAFIIFWVRLKIQVRKAAITSYEKSDGVYTGLSTRNQETYETLKHEKPPQGSGATNFSLLKQAGDVEENPGPMWQLLLPTALLLLVSAGMRTEDLPKAVVFLEPQWYRVLEKDSVTLKCQGAYSPEDNSTQWFHNESLISSQASSYFIDAATVDDSGEYRCQTNLSTLSDPVQLEVHIGWLLLQAPRWVFKEEDPIHLRCHSWKNTALHKVTYLQNGKGRKYFHHNSDFYIPKATLKDSGSYFCRGLVGSKNVSSETVNITITQGLAVSTISSFFPPGYQVSFCLVMVLLFAVDTGLYFSVKTNIRSSTRDWKDHKFKWRKDPQDK

SEQ ID NO: 30 - protein, 160 aa, synthetic construct; identical to SEQ ID NO: 22
  REGION 1..160: note = ERIL-2 protein

SEQ ID NO: 31 - DNA, 3126 bp, synthetic construct
  misc_feature 1..3126: note = Codon-optimized CD33ScfV-P2A-CD16-IRES-erIL2
  source 1..3126: mol_type = other DNA
atggactggatctggcgcatcctcttcctcgtcggcgctgctaccggcgctcattcggcccagccggccgacattcaaatgactcagtccccttccagcttgtcagcctcagtaggggaccgggtcacgatcacctgtcgagcgtctgagtcagtggataactacgggatttctttcatgaactggttccagcagaagcccggcaaagctcctaagctccttatatatgcagcctcaaatcaggggagcggtgttcctagtcgcttcagtggaagcggtagcggtacggactttacgttgacgataagtagccttcagccagatgactttgccacttattattgtcagcagtctaaggaagttccttggacgtttggccaaggaacgaaggtcgaaatcaaagggggagggggctcaggagggggcggcagtggtggtggaggctctcaagtccaactcgtacagtctggcgcggaggttaaaaagccgggaagctccgtgaaagtatcctgtaaggcaagcggatacacctttaccgattataacatgcactgggttaggcaggcgcccggccaaggtctggaatggatcggttatatttatccatacaacggtggtaccggctataatcagaagtttaagagtaaggctactattacagcggatgagtcaaccaatactgcatacatggagctctcctcactcaggagcgaagataccgcagtgtattactgtgcccgagggagaccagccatggactactggggtcagggtacccttgtgacagtatctagcgcggccgcgctgagcaacagcatcatgtacttcagccacttcgtgcctgtgttcctgcctgccaagcctacaacaacaccagcccctagacctccaacccctgcccctacaattgcctctcagcctctgtctctgaggcccgaagcttgtagacctgctgctggcggagctgtgcacaccagaggactggatttcgcctgcttttgggtgctggtggtcgtgggcggagtgctggcttgttattctctgctggtcaccgtggccttcatcatcttttgggtccgactgaagatccaggtccgaaaggccgccatcaccagctacgagaagtctgatggcgtgtacaccggcctgagcaccagaaaccaggaaacctacgagacactgaagcacgagaagcccccccagggaagcggagctactaacttcagcctgctgaagcaggctggagacgtggaggagaaccctggacctatgtggcagctgctgctgcctacagctctcctgctgctggtgtccgccggcatgagaaccgaggatctgcctaaggccgtggtgttcctggaaccccagtggtacagagtgctggaaaaggacagcgtgaccctgaagtgccagggcgcctacagccccgaggacaatagcacccagtggttccacaacgagagcctgatcagcagccaggccagcagctacttcatcgacgccgccaccgtggacgacagcggcgagtatagatgccagaccaacctgagcaccctgagcgaccccgtgcagctggaagtgcacatcggatggctgctgctgcaggcccccagatgggtgttcaaagaagaggaccccatccacctgagatgccactcttggaagaacaccgccctgcacaaagtgacctacctgcagaacggcaagggcagaaagtacttccaccacaacagcgacttctacatccccaaggccaccctgaaggactccggctcctacttctgcagaggcctcgtgggcagcaagaacgtgtccagcgagacagtgaacatcaccatcacccagggcctggccgtgtctaccatcagcagctttttcccacccggctaccaggtgtccttctgcctcgtgatggtgctgctgttcgccgtggacaccggcctgtacttcagcgtgaaaacaaacatcagaagcagcacccgggactggaaggaccacaagttcaagtggcggaaggacccccaggacaagtgaaattccgcccctctcccccccccccctctccctcccccccccctaacgttactggccgaagccgcttggaataaggccggtgtgcgtttgtctatatgttattttccaccatattgccgtcttttggcaatgtgagggcccggaaacctggccctgtcttcttgacgagcattcctaggggtctttcccctctcgccaaaggaatgcaaggtctgttgaatgtcgtgaaggaagcagttcctctggaagcttcttgaagacaaacaacgtctgtagcgaccctttgcaggcagcggaaccccccacctggcgacaggtgcctctgcggccaaaagccacgtgtataagatacacctgcaaaggcggcacaaccccagtgccacgttgtgagttggatagttgtggaaagagtcaaatggctctcctcaagcgtattcaacaaggggctgaaggatgcccagaaggtaccccattgtatgggatctgatctggggcctcggtgcacatgctttacatgtgtttagtcgaggttaaaaaaacgtctaggccccccgaaccacggggacgtggttttcctttgaaaaacacgataaccgccaccatgtaccggatgcagctgctgagctgtatcgccctgtctctggccctcgtgaccaacagcgcccctaccagcagcagcaccaagaaaacccagctgcagctggaacatctgctgctggacctgcagatgatcctgaacggcatcaacaactacaagaaccccaagctgacccggatgctgaccttcaagttctacatgcccaagaaggccaccgaactgaaacatctgcagtgcctggaagaggaactgaagcccctggaagaagtgctgaacctggcccagagcaagaacttccacctgaggcccagggacctgatcagcaacatcaacgtgatcgtgctggaactgaaaggcagcgagacaaccttcatgtgcgagtacgccgacgagacagctaccatcgtggaatttctgaaccggtggatcaccttctgccagagcatcatcagcaccctgaccggctccgagaaggacgagctgtgagcggccgc

SEQ ID NO: 32 - protein, 677 aa, synthetic construct
  REGION 1..677: note = CD33 CAR-P2A-CD16 peptide
MDWIWRILFLVGAATGAHSAQPADIQMTQSPSSLSASVGDRVTITCRASESVDNYGISFMNWFQQKPGKAPKLLIYAASNQGSGVPSRFSGSGSGTDFTLTISSLQPDDFATYYCQQSKEVPWTFGQGTKVEIKGGGGSGGGGSGGGGSQVQLVQSGAEVKKPGSSVKVSCKASGYTFTDYNMHWVRQAPGQGLEWIGYIYPYNGGTGYNQKFKSKATITADESTNTAYMELSSLRSEDTAVYYCARGRPAMDYWGQGTLVTVSSAAALSNSIMYFSHFVPVFLPAKPTTTPAPRPPTPAPTIASQPLSLRPEACRPAAGGAVHTRGLDFACFWVLVVVGGVLACYSLLVTVAFIIFWVRLKIQVRKAAITSYEKSDGVYTGLSTRNQETYETLKHEKPPQGSGATNFSLLKQAGDVEENPGPMWQLLLPTALLLLVSAGMRTEDLPKAVVFLEPQWYRVLEKDSVTLKCQGAYSPEDNSTQWFHNESLISSQASSYFIDAATVDDSGEYRCQTNLSTLSDPVQLEVHIGWLLLQAPRWVFKEEDPIHLRCHSWKNTALHKVTYLQNGKGRKYFHHNSDFYIPKATLKDSGSYFCRGLVGSKNVSSETVNITITQGLAVSTISSFFPPGYQVSFCLVMVLLFAVDTGLYFSVKTNIRSSTRDWKDHKFKWRKDPQDK

SEQ ID NO: 33 - protein, 192 aa, synthetic construct
  REGION 1..192: note = erIL2
MLYMCLVEVKKTSRPPEPRGRGFPLKNTITATMYRMQLLSCIALSLALVTNSAPTSSSTKKTQLQLEHLLLDLQMILNGINNYKNPKLTRMLTFKFYMPKKATELKHLQCLEEELKPLEEVLNLAQSKNFHLRPRDLISNINVIVLELKGSETTFMCEYADETATIVEFLNRWITFCQSIISTLTGSEKDEL

SEQ ID NO: 34 - protein, 254 aa, synthetic construct
  REGION 1..254: note = sp|P08637|FCG3A_HUMAN Low affinity IgG gamma FcR III-A
MWQLLLPTALLLLVSAGMRTEDLPKAVVFLEPQWYRVLEKDSVTLKCQGAYSPEDNSTQWFHNESLISSQASSYFIDAATVDDSGEYRCQTNLSTLSDPVQLEVHIGWLLLQAPRWVFKEEDPIHLRCHSWKNTALHKVTYLQNGKGRKYFHHNSDFYIPKATLKDSGSYFCRGLFGSKNVSSETVNITITQGLAVSTISSFFPPGYQVSFCLVMVLLFAVDTGLYFSVKTNIRSSTRDWKDHKFKWRKDPQDK

SEQ ID NO: 35 - protein, 254 aa, synthetic construct
  REGION 1..254: note = High Affinity Variant Immunoglobulin Gamma FcRIII-A
MWQLLLPTALLLLVSAGMRTEDLPKAVVFLEPQWYRVLEKDSVTLKCQGAYSPEDNSTQWFHNESLISSQASSYFIDAATVDDSGEYRCQTNLSTLSDPVQLEVHIGWLLLQAPRWVFKEEDPIHLRCHSWKNTALHKVTYLQNGKGRKYFHHNSDFYIPKATLKDSGSYFCRGLVGSKNVSSETVNITITQGLAVSTISSFFPPGYQVSFCLVMVLLFAVDTGLYFSVKTNIRSSTRDWKDHKFKWRKDPQDK

SEQ ID NO: 36 - DNA, 765 bp, synthetic construct
  misc_feature 1..765: note = High Affinity Variant Ig Gamma Fc Region Receptor III-A DNA
  source 1..765: mol_type = other DNA
atgtggcagctgctgctgcctacagctctcctgctgctggtgtccgccggcatgagaaccgaggatctgcctaaggccgtggtgttcctggaaccccagtggtacagagtgctggaaaaggacagcgtgaccctgaagtgccagggcgcctacagccccgaggacaatagcacccagtggttccacaacgagagcctgatcagcagccaggccagcagctacttcatcgacgccgccaccgtggacgacagcggcgagtatagatgccagaccaacctgagcaccctgagcgaccccgtgcagctggaagtgcacatcggatggctgctgctgcaggcccccagatgggtgttcaaagaagaggaccccatccacctgagatgccactcttggaagaacaccgccctgcacaaagtgacctacctgcagaacggcaagggcagaaagtacttccaccacaacagcgacttctacatccccaaggccaccctgaaggactccggctcctacttctgcagaggcctcgtgggcagcaagaacgtgtccagcgagacagtgaacatcaccatcacccagggcctggccgtgtctaccatcagcagctttttcccacccggctaccaggtgtccttctgcctcgtgatggtgctgctgttcgccgtggacaccggcctgtacttcagcgtgaaaacaaacatcagaagcagcacccgggactggaaggaccacaagttcaagtggcggaaggacccccaggacaagtga

SEQ ID NO: 37 - DNA, 1233 bp, synthetic construct
  misc_feature 1..1233: note = artificial sequence
  source 1..1233: mol_type = other DNA
atggactggatctggcggattctgtttctcgtgggagctgccacaggcgctcattctgctcagcctgccgacatccagatgacccagagccccagcagcctgagcgccagcgtgggcgacagagtgaccatcacctgcagagccagccaggacgtgaacaccgccgtggcctggtaccagcagaagcccggcaaggcccccaagctgctgatctacagcgccagcttcctgtacagcggcgtgcccagcagattcagcggcagcagaagcggcaccgacttcaccctgaccatcagcagcctgcagcccgaggacttcgccacctactactgccagcagcactacaccaccccccccaccttcggccagggcaccaaggtggagatcaagtcctcagggggcgggggaagtggtgggggcggcagcggcggagggggctcaggaggaggcggatcaggcggatcagaggtgcagctggtggagagcggcggcggcctggtgcagcccggcggcagcctgagactgagctgcgccgccagcggcttcaacatcaaggacacctacatccactgggtgagacaggcccccggcaagggcctggagtgggtggccagaatctaccccaccaacggctacaccagatacgccgacagcgtgaagggcagattcaccatcagcgccgacaccagcaagaacaccgcctacctgcagatgaacagcctgagagccgaggacaccgccgtgtactactgcagcagatggggcggcgacggcttctacgccatggactactggggccagggcaccctggtgaccgtgagcagcgcggccgcgctgagcaacagcatcatgtacttcagccacttcgtgcctgtgttcctgcctgccaagcctacaacaacaccagcccctagacctccaacccctgcccctacaattgcctctcagcctctgtctctgaggcccgaagcttgtagacctgctgctggcggagctgtgcacaccagaggactggatttcgcctgcttttgggtgctggtggtcgtgggcggagtgctggcttgttattctctgctggtcaccgtggccttcatcatcttttgggtccgactgaagatccaggtccgaaaggccgccatcaccagctacgagaagtctgatggcgtgtacaccggcctgagcaccagaaaccaggaaacctacgagacactgaagcacgagaagcccccccag

SEQ ID NO: 38 - DNA, 1230 bp, synthetic construct
  misc_feature 1..1230: note = artificial sequence
  source 1..1230: mol_type = other DNA
atggactggatctggcggattctgtttctcgtgggagctgccacaggcgctcattctgctcagcctgccgatatccaaatgactcaatctcctagttcactgtcagcctctgttggtgatcgcgtgaccattacctgccaagctagccaggatattagcaactacttgaactggtatcagcagaagcctggcaaagccccaaagctgttgatctacgatgtaagtaacttggaaactggcgtcccaagccgcttctctggatctggttcaggcaccgacttcactttcactatcagcagcctgcagcctgaagatatcgcaacctactattgccagcaggttgctaatgttcctctgactttcggccaaggcaccaaggtggagatcaagggcggcggaggaagcggaggcggaggatctgggggcggaggctctggcggagggggatctgaagttcagcttgtagaatctggaggtggattggttcaacctggtggctctcttcgcctgagttgtgcagcctctggttttactttctctagttactggatgcattgggttcgtcaggctcctgggaaaggcctggaatgggtttcagctattagttggagtggagatagtacttactacgcagacagtgtgaaaggtcgcttcaccatcagccgtgataattctaagaacactttgtacctgcaaatgaactccttgcgcgcagaagacacggctgtgtactattgtgcccgtgatcgctctgcgacttggtattatctggggcttggtttcgatgtatggggacaaggtaccctggtaacggtttctagcgcggccgcgctgagcaacagcatcatgtacttcagccacttcgtgcctgtgttcctgcctgccaagcctacaacaacaccagcccctagacctccaacccctgcccctacaattgcctctcagcctctgtctctgaggcccgaagcttgtagacctgctgctggcggagctgtgcacaccagaggactggatttcgcctgcttttgggtgctggtggtcgtgggcggagtgctggcttgttattctctgctggtcaccgtggccttcatcatcttttgggtccgactgaagatccaggtccgaaaggccgccatcaccagctacgagaagtctgatggcgtgtacaccggcctgagcaccagaaaccaggaaacctacgagacactgaagcacgagaagcccccccag

SEQ ID NO: 39 - DNA, 1215 bp, synthetic construct
  misc_feature 1..1215: note = artificial sequence
  source 1..1215: mol_type = other DNA
atggactggatctggcggattctgtttctcgtgggagctgccacaggcgctcattctgctcagcctgccgatattcttcttactcaatctcccgttattttgtcagtatccccaggtgagcgagtcagcttctcttgtcgagcgtcacaatccattggcaccaacatacattggtaccaacagcgcaccaacgggtctccccggctcttgattaagtacgcatcagaaagtatttctgggatacccagtaggttctcagggagcgggagtggcactgactttaccctgtccataaacagcgttgagtctgaggacatcgcggactactattgtcagcagaacaacaattggccgaccacgtttggtgcgggaacaaaacttgaactcaaaggcggcggaggaagcggaggcggaggatctgggggcggaggctctggcggagggggatctcaggtgcagctcaaacagtcaggacctggcctcgttcagccaagccaatcactgagtataacgtgcacggtgagcggctttagcctgacaaactatggtgtccactgggtccgccaatctcctggaaaaggcttggagtggctcggtgttatctggtccggtggtaacacagactacaacacgccattcaccagtcgccttagtattaacaaggacaactccaagtctcaggttttctttaaaatgaactctctgcagtctaatgataccgcaatttactactgtgcgagggcactcacgtactatgactatgagttcgcgtattggggccaagggactctcgttactgtctcagcggcggccgcgctgagcaacagcatcatgtacttcagccacttcgtgcctgtgttcctgcctgccaagcctacaacaacaccagcccctagacctccaacccctgcccctacaattgcctctcagcctctgtctctgaggcccgaagcttgtagacctgctgctggcggagctgtgcacaccagaggactggatttcgcctgcttttgggtgctggtggtcgtgggcggagtgctggcttgttattctctgctggtcaccgtggccttcatcatcttttgggtccgactgaagatccaggtccgaaaggccgccatcaccagctacgagaagtctgatggcgtgtacaccggcctgagcaccagaaaccaggaaacctacgagacactgaagcacgagaagcccccccag

SEQ ID NO: 40 - DNA, 1230 bp, synthetic construct
  misc_feature 1..1230: note = artificial sequence
  source 1..1230: mol_type = other DNA
atggactggatctggcggattctgtttctcgtgggagctgccacaggcgctcattctgctcagcctgccgatgttgtaatgacgcagtcacccctgtcactcccggtcacacccggagaaccagcgtcaattagctgccgatctagccaaagtttgcttcattccaatggttacaattatctcgactggtacttgcagaaacccggccaatcccctcagctgctcatctaccttgggtctaatagggcatctggggttcccgataggttctctggctccgggagcggcaccgactttacgttgaaaatctctagggttgaggcggaagacgtaggcgtttactattgcatgcaggggacccactggccgctgaccttcggccagggcaccaaggttgaaataaaaggcggcggaggaagcggaggcggaggatctgggggcggaggctctggcggagggggatctcaggtacagctccaggaatcaggacccggtttggttaagccctccgggaccctttccctcacgtgtgcagtctcaggtgggtcaattagttcttccaattggtggtcttgggtgcggcaaccacctggtaaaggtctcgagtggataggggaaatttatcatagtggctccaccaattataacccctcactcaagtccagggttacgatatctgtggacaaaagtaaaaaccaattctccctcaaacttagtagtgtaacagcggcagacaccgcggtgtactactgcgcacggtggacaggccgaactgatgcctttgacatttggggacagggaactatggtgactgtgtcatccgcggccgcgctgagcaacagcatcatgtacttcagccacttcgtgcctgtgttcctgcctgccaagcctacaacaacaccagcccctagacctccaacccctgcccctacaattgcctctcagcctctgtctctgaggcccgaagcttgtagacctgctgctggcggagctgtgcacaccagaggactggatttcgcctgcttttgggtgctggtggtcgtgggcggagtgctggcttgttattctctgctggtcaccgtggccttcatcatcttttgggtccgactgaagatccaggtccgaaaggccgccatcaccagctacgagaagtctgatggcgtgtacaccggcctgagcaccagaaaccaggaaacctacgagacactgaagcacgagaagcccccccag

SEQ ID NO: 41 - DNA, 1203 bp, synthetic construct
  misc_feature 1..1203: note = artificial sequence
  source 1..1203: mol_type = other DNA
atggactggatctggcgcatcctcttcctcgtcggcgctgctaccggcgctcattcggcccagccggccgacattcaaatgactcagtccccttccagcttgtcagcctcagtaggggaccgggtcacgatcacctgtcgagcgtctgagtcagtggataactacgggatttctttcatgaactggttccagcagaagcccggcaaagctcctaagctccttatatatgcagcctcaaatcaggggagcggtgttcctagtcgcttcagtggaagcggtagcggtacggactttacgttgacgataagtagccttcagccagatgactttgccacttattattgtcagcagtctaaggaagttccttggacgtttggccaaggaacgaaggtcgaaatcaaagggggagggggctcaggagggggcggcagtggtggtggaggctctcaagtccaactcgtacagtctggcgcggaggttaaaaagccgggaagctccgtgaaagtatcctgtaaggcaagcggatacacctttaccgattataacatgcactgggttaggcaggcgcccggccaaggtctggaatggatcggttatatttatccatacaacggtggtaccggctataatcagaagtttaagagtaaggctactattacagcggatgagtcaaccaatactgcatacatggagctctcctcactcaggagcgaagataccgcagtgtattactgtgcccgagggagaccagccatggactactggggtcagggtacccttgtgacagtatctagcgcggccgcgctgagcaacagcatcatgtacttcagccacttcgtgcctgtgttcctgcctgccaagcctacaacaacaccagcccctagacctccaacccctgcccctacaattgcctctcagcctctgtctctgaggcccgaagcttgtagacctgctgctggcggagctgtgcacaccagaggactggatttcgcctgcttttgggtgctggtggtcgtgggcggagtgctggcttgttattctctgctggtcaccgtggccttcatcatcttttgggtccgactgaagatccaggtccgaaaggccgccatcaccagctacgagaagtctgatggcgtgtacaccggcctgagcaccagaaaccaggaaacctacgagacactgaagcacgagaagcccccccag

SEQ ID NO: 42 - DNA, 1215 bp, synthetic construct
  misc_feature 1..1215: note = artificial sequence
  source 1..1215: mol_type = other DNA
atggactggatctggcggattctgtttctcgtgggagctgccacaggcgctcattctgctcagcctgccaacatccagatgacccagtctccatcttctgtgtctgcatctgtaggagacagagtcaccatcacttgtcgggcgagtcaggatattagccgctggttagcctggtatcagcagaaaccagggaaagcccctaaactcctgatctatgctgcatccagtttgcaaagtggggtcccatcgaggttcagcggcagtggatctgggacagatttcgctctcactatcagcagcctgcagcctgaagattttgcaacttactattgtcaacaggctgacagtcgtttctcgatcaccttcggccaagggacacgactggagattaaaggcggcggaggaagcggaggcggaggatctgggggcggaggctctggcggagggggatctgaggtgcagctggtgcagtctgggggaggcttggtacagcctggggggtccctgagactctcctgtgcagcctctggattcaccttcagtagctatagcatgaactgggtccgccaggctccagggaaggggctggagtgggtttcatacattagtagtagtagtagtaccatacagtacgcagactctgtgaagggccgattcaccatctccagagacaatgccaagaactcactgtatctgcaaatgaacagcctgagagacgaggacacggctgtgtattactgtgcgagaggggactactactacggtatggacgtctggggccaagggaccacggtcaccgtgagctcagcggccgcgctgagcaacagcatcatgtacttcagccacttcgtgcctgtgttcctgcctgccaagcctacaacaacaccagcccctagacctccaacccctgcccctacaattgcctctcagcctctgtctctgaggcccgaagcttgtagacctgctgctggcggagctgtgcacaccagaggactggatttcgcctgcttttgggtgctggtggtcgtgggcggagtgctggcttgttattctctgctggtcaccgtggccttcatcatcttttgggtccgactgaagatccaggtccgaaaggccgccatcaccagctacgagaagtctgatggcgtgtacaccggcctgagcaccagaaaccaggaaacctacgagacactgaagcacgagaagcccccccag

SEQ ID NO: 43 - DNA, 1203 bp, synthetic construct; identical to SEQ ID NO: 41
  misc_feature 1..1203: note = artificial sequence
  source 1..1203: mol_type = other DNA

SEQ ID NO: 44 - DNA, 1596 bp, synthetic construct
  misc_feature 1..1596: note = artificial sequence
  source 1..1596: mol_type = other DNA
atgaaccggggagtcccttttaggcacttgcttctggtgctgcaactggcgctcctcccagcagccactcagggaaagaaagtggtgctgggcaaaaaaggggatacagtggaactgacctgtacagcttcccagaagaagagcatacaattccactggaaaaactccaaccagataaagattctgggaaatcagggctccttcttaactaaaggtccatccaagctgaatgatcgcgctgactcaagaagaagcctttgggaccaaggaaactttcccctgatcatcaagaatcttaagatagaagactcagatacttacatctgtgaagtggaggaccagaaggaggaggtgcaattgctagtgttcggattgactgccaactctgacacccacctgcttcaggggcagagcctgaccctgaccttggagagcccccctggtagtagcccctcagtgcaatgtaggagtccaaggggtaaaaacatacagggggggaagaccctctccgtgtctcagctggagctccaggatagtggcacctggacatgcactgtcttgcagaaccagaagaaggtggagttcaaaatagacatcgtggtgctagctttccagaaggcctccagcatagtctataagaaagagggggaacaggtggagttctccttcccactcgcctttacagttgaaaagctgacgggcagtggcgagctgtggtggcaggcggagagggcttcctcctccaagtcttggatcacctttgacctgaagaacaaggaagtgtctgtaaaacgggttacccaggaccctaagctccagatgggcaagaagctcccgctccacctcaccctgccccaggccttgcctcagtatgctggctctggaaacctcaccctggcccttgaagcgaaaacaggaaagttgcatcaggaagtgaacctggtggtgatgagagccactcagctccagaaaaatttgacctgtgaggtgtggggacccacctcccctaagctgatgctgagtttgaaactggagaacaaggaggcaaaggtctcgaagcgggagaaggcggtgtgggtgctgaaccctgaggcggggatgtggcagtgtctgctgagtgactcgggacaggtcctgctggaatccaacatcaaggttctgcccacatggtccaccccggtgcagccagcggccgcgctgagcaacagcatcatgtacttcagccacttcgtgcctgtgttcctgcctgccaagcctacaacaacaccagcccctagacctccaacccctgcccctacaattgcctctcagcctctgtctctgaggcccgaagcttgtagacctgctgctggcggagctgtgcacaccagaggactggatttcgcctgcttttgggtgctggtggtcgtgggcggagtgctggcttgttattctctgctggtcaccgtggccttcatcatcttttgggtccgactgaagatccaggtccgaaaggccgccatcaccagctacgagaagtctgatggcgtgtacaccggcctgagcaccagaaaccaggaaacctacgagacactgaagcacgagaagcccccccag

SEQ ID NO: 45 - DNA, 1215 bp, synthetic construct
  misc_feature 1..1215: note = artificial sequence
  source 1..1215: mol_type = other DNA
atggactggatctggcggattctgtttctcgtgggagctgccacaggcgctcattctgctcagcctgccgaagttcagcttgtagaatctggaggtggattggttcaacctggtggctctcttcgcctgagttgtgcagcctctggttttactttcaatagttacgctatgcattgggttcgtcaggctcctgggaaaggcctggaatgggtttcagctattagtggtaatggaggtagtactcgttacgcagacagtgtgaaaggtcgcttcaccatcagccgtgataattctaagaacactttgtacctgcaaatgaactccttgcgcgcagaagacacggctgtgtactattgtgcccgtgatcgctttcggaaggttcatggtttcgatgtatggggacaaggtaccctggtaacggtttctagcggaggtggtgggagtggtggaggcggctcgggtggaggtggttcaggaggaggcggagatatccaaatgactcaatctcctagttcactgtcagcctctgttggtgatcgcgtgaccattacctgccaagctagccaggatattagcaactacttgaactggtatcagcagaagcctggcaaagccccaaagctgttgatctacgatgcaagtaacttggaaactggcgtcccaagccgcttctctggatctggttcaggcaccgacttcactttcactatcagcagcctgcagcctgaagatatcgcaacctactattgccagcaggatgctacttttcctttgactttcggccaaggcaccaaggtggagatcaaggcggccgcgctgagcaacagcatcatgtacttcagccacttcgtgcctgtgttcctgcctgccaagcctacaacaacaccagcccctagacctccaacccctgcccctacaattgcctctcagcctctgtctctgaggcccgaagcttgtagacctgctgctggcggagctgtgcacaccagaggactggatttcgcctgcttttgggtgctggtggtcgtgggcggagtgctggcttgttattctctgctggtcaccgtggccttcatcatcttttgggtccgactgaagatccaggtccgaaaggccgccatcaccagctacgagaagtctgatggcgtgtacaccggcctgagcaccagaaaccaggaaacctacgagacactgaagcacgagaagcccccccag

SEQ ID NO: 46 - DNA, 1194 bp, synthetic construct
  misc_feature 1..1194: note = artificial sequence
  source 1..1194: mol_type = other DNA
atggactggatctggcggattctgtttctcgtgggagctgccacaggcgctcattctgctcagcctgccgtccagctgcagcagtctggacctgagctggtaaagcctggggcttcagtgaagatgtcctgcaaggcttctggatacacattcactagctatgttatgcactgggtgaagcagaagcctgggcagggccttgagtggattggatatattattccttacaatgatgctactaagtacaatgagaagttcaaaggcaaggccacactgacttcagacaaatcctccagcacagcctacatggagctcagcagcctgacctctgaggactctgcggtctattactgtgcacgctataattacgacgggtacttcgatgtctggggcgcagggaccacggtcaccgtctcctcaggcggcggaggaagcggaggcggaggatctgggggcggaggctctgacattgtgatgactcagtctccagccaccctgtctgtgactccaggagatagagtctctctttcctgcagggccagccagagtattagcgactacttacactggtatcaacaaaaatcacatgagtctccaaggcttctcatcaaatatgcttcccaatccatctctggaatcccctccaggttcagtggcagtggatcagggtcagatttcactctcagtatcaacagtgtggaacctgaagatgttggagtgtattactgtcaaaatggtcacagctttcctccgacgttcggtggaggcaccaagctggaaatcaaagcggccgcgctgagcaacagcatcatgtacttcagccacttcgtgcctgtgttcctgcctgccaagcctacaacaacaccagcccctagacctccaacccctgcccctacaattgcctctcagcctctgtctctgaggcccgaagcttgtagacctgctgctggcggagctgtgcacaccagaggactggatttcgcctgcttttgggtgctggtggtcgtgggcggagtgctggcttgttattctctgctggtcaccgtggccttcatcatcttttgggtccgactgaagatccaggtccgaaaggccgccatcaccagctacgagaagtctgatggcgtgtacaccggcctgagcaccagaaaccaggaaacctacgagacactgaagcacgagaagcccccccag

SEQ ID NO: 47 - DNA, 1206 bp, synthetic construct
  misc_feature 1..1206: note = artificial sequence
  source 1..1206: mol_type = other DNA
atggactggatctggcggattctgtttctcgtgggagctgccacaggcgctcattctgctcagcctgcccaggtgcaagtgaaagagtctggccctggactggtggccccaagccagtctctgagcatcacatgtaccgtgtccggcttcagcctgaccaactatggcgtgcactgggtccgacagcctccaggcaaaggactggaatggctgggagtgatttgggctggcggcagcaccaactacaacagcgccctgatgagccggctgagcatctccaaggacaacagcaagagccaggtgttcctgaagatgaacagcctgcagaccgacgacaccgccatgtactactgtgctagcagaggcggcaactacggctacgccctggattattggggccagggcacaagcgtgaccgtgtcatctggcggcggaggaagcggaggcggaggatctgggggcggaggctctggcggagggggatctagcatcgtgatgacccagactcctaagttcctgctggtgtctgccggcgacagagtgaccatcacctgtaaagccagccagagcgtgtccaacgacgtggcctggtatcagcagaagcctggacagagccccaagctgctgatctacagcgccagcaacagatacaccggcgtgcccgatagattcaccggctctggctacggcaccgacttcacctttaccatcagcaccgtgcaggccgaggatctggccgtgtacttctgccagcaagactacagctctctcggcggaggcaccaagctggaaatcaaagcggccgcgctgagcaacagcatcatgtacttcagccacttcgtgcctgtgttcctgcctgccaagcctacaacaacaccagcccctagacctccaacccctgcccctacaattgcctctcagcctctgtctctgaggcccgaagcttgtagacctgctgctggcggagctgtgcacaccagaggactggatttcgcctgcttttgggtgctggtggtcgtgggcggagtgctggcttgttattctctgctggtcaccgtggccttcatcatcttttgggtccgactgaagatccaggtccgaaaggccgccatcaccagctacgagaagtctgatggcgtgtacaccggcctgagcaccagaaaccaggaaacctacgagacactgaagcacgagaagcccccccag

SEQ ID NO: 48 - DNA, 1248 bp, synthetic construct
  misc_feature 1..1248: note = artificial sequence
  source 1..1248: mol_type = other DNA
atggactggatctggcggattctgtttctcgtgggagctgccacaggcgctcattctgctcagcctgcccaggttcagctgcagcagtctggacctgagctggttaagcctggcgcctccgtgaagatgagctgcaagaccagccggtacaccttcaccgagtacaccatccactgggtccgacagagccacggcaagagcctggaatggatcggcggcatcaaccccaacaacggcatccccaactacaaccagaagttcaagggcagagccacactgaccgtgggcaagtctagcagcaccgcctacatggaactgcggagcctgacaagcgaggacagcgccgtgtacttctgcgccagaagaagaatcgcctacggctacgatgagggccacgccatggattattggggccagggaacaagcgtgaccgtgtctagtggcggcggaggaagcggaggcggaggatctgggggcggaggctctggcggagggggatctgacatcgtgatgacacagagcccttctagcctggccgtgtccgtgggagagaaagtgaccatgagctgcaagagcagccagagcctgctgtactcccggaaccagaagaactacctggcctggttccagcagaagcccggccagtctcctaagctgctgatcttctgggccagcaccagagaaagcggcgtgcccgatagattcaccggcagcggctttggcaccgacttcaacctgacaatcagcagcgtgcaggccgaggacctggctgtgtacgattgccagcagtacttcagctaccctctgacctttggagccggcaccaagctggaactgagagcggccgcgctgagcaacagcatcatgtacttcagccacttcgtgcctgtgttcctgcctgccaagcctacaacaacaccagcccctagacctccaacccctgcccctacaattgcctctcagcctctgtctctgaggcccgaagcttgtagacctgctgctggcggagctgtgcacaccagaggactggatttcgcctgcttttgggtgctggtggtcgtgggcggagtgctggcttgttattctctgctggtcaccgtggccttcatcatcttttgggtccgactgaagatccaggtccgaaaggccgccatcaccagctacgagaagtctgatggcgtgtacaccggcctgagcaccagaaaccaggaaacctacgagacactgaagcacgagaagcccccccag

SEQ ID NO: 49 - DNA, 510 bp, synthetic construct
  misc_feature 1..510: note = artificial sequence
  source 1..510: mol_type = other DNA
atgcgcatcagcaagccccacctgcgcagcatcagcatccagtgctacctgtgcctgctgctgaacagccacttcctgaccgaggccggcatccacgtgttcatcctgggctgcttcagcgccggcctgcccaagaccgaggccaactgggtgaacgtgatcagcgacctgaagaagatcgaggacctgatccagagcatgcacatcgacgccaccctgtacaccgagagcgacgtgcaccccagctgcaaggtgaccgccatgaagtgcttcctgctggagctgcaggtgatcagcctggagagcggcgacgccagcatccacgacaccgtggagaacctgatcatcctggccaacaacagcctgagcagcaacggcaacgtgaccgagagcggctgcaaggagtgcgaggagctggaggagaagaacatcaaggagttcctgcagagcttcgtgcacatcgtgcagatgttcatcaacaccagcggctccgagaaggacgagctgtaa

SEQ ID NO: 50 - protein, 169 aa, synthetic construct
  REGION 1..169: note = artificial sequence
MRISKPHLRSISIQCYLCLLLNSHFLTEAGIHVFILGCFSAGLPKTEANWVNVISDLKKIEDLIQSMHIDATLYTESDVHPSCKVTAMKCFLLELQVISLESGDASIHDTVENLIILANNSLSSNGNVTESGCKECEELEEKNIKEFLQSFVHIVQMFINTSGSEKDEL

SEQ ID NO: 51 - DNA, 1215 bp, synthetic construct
  misc_feature 1..1215: note = artificial sequence
  source 1..1215: mol_type = other DNA
atggactggatctggcgcatcctcttcctcgtcggcgctgctaccggcgctcattcggcccagccggccatggcgcaagtaaaactccaagaatctggggcggagctggtgaaaccgggggcgtctgtgaagatgagctgtaaagcatcaggctacaccttcacctcctataatatgcactgggtgaaacaaacacccggacagggcctcgaatggattggtgccatctatcctggaaatggtgatacctcatataatcagaagtttaagggcaaggctacgcttactgcggataaaagctcttccactgcttacatgcaactgagcagtctcacttcagaggactcagccgattattattgtgcccgcagcaactactatggtagttcatactggtttttcgacgtttgggggcaaggtaccaccgtcacggtttcttctggtgggggcggaagcgggggtggaggatctgggggcggtggttcagacattgaactcacccagagccctactattctgagcgcgtctccaggtgaaaaagttacgatgacgtgcagagcatcaagtagtgtgaattatatggattggtatcaaaagaagccaggctcatccccaaaaccgtggatctatgcaactagcaacctcgcgtcaggggtgccagcaaggttttccggaagtggttctggcacatcttatagtctcaccatttcccgagtggaggctgaggatgcggccacttattactgccagcaatggtcattcaatcccccaacatttggtggcggaacaaaactcgaaattaaacgggcggccgcgctgagcaacagcatcatgtacttcagccacttcgtgcctgtgttcctgcctgccaagcctacaacaacaccagcccctagacctccaacccctgcccctacaattgcctctcagcctctgtctctgaggcccgaagcttgtagacctgctgctggcggagctgtgcacaccagaggactggatttcgcctgcttttgggtgctggtggtcgtgggcggagtgctggcttgttattctctgctggtcaccgtggccttcatcatcttttgggtccgactgaagatccaggtccgaaaggccgccatcaccagctacgagaagtctgatggcgtgtacaccggcctgagcaccagaaaccaggaaacctacgagacactgaagcacgagaagcccccccag

SEQ ID NO: 52 - DNA, 1248 bp, synthetic construct
  misc_feature 1..1248: note = artificial sequance
  source 1..1248: mol_type = other DNA
atggactggatctggcgcatcctcttcctcgtcggcgctgctaccggcgctcattcggcccagccggccgatatcgagctcacccaatctccaaaattcatgtccacatcagtaggagacagggtcagcgtcacctgcaaggccagtcagaatgtggatactaatgtagcgtggtatcaacaaaaaccagggcaatctcctgaaccactgcttttctcggcatcctaccgttacactggagtccctgatcgcttcacaggcagtggatctgggacagatttcactctcaccatcagcaatgtgcagtctgaagacttggcagagtatttctgtcagcaatataacagctatcctctgacgttcggtggcggcaccaagctggaaatcaaacgggctgccgcagaaggtggaggcggttcaggtggcggaggttccggcggaggtggctctggcggtggcggatcggccatggcccaggtgaagctgcagcagtcaggagggggcttggtgcaacctggaggctccatgaaactctcctgtgttgtctctggattcactttcagtaattactggatgaactgggtccgccagtctccagagaaggggcttgagtggattgcagaaattagattgaaatccaataattttggaagatattatgcggagtctgtgaaagggaggttcaccatctcaagagatgattccaaaagtagtgcctacctgcaaatgatcaacctaagagctgaagatactggcatttattactgtaccagttatggtaactacgttgggcactattttgaccactggggccaagggaccacggtcaccgtatcgagtgcggccgcgctgagcaacagcatcatgtacttcagccacttcgtgcctgtgttcctgcctgccaagcctacaacaacaccagcccctagacctccaacccctgcccctacaattgcctctcagcctctgtctctgaggcccgaagcttgtagacctgctgctggcggagctgtgcacaccagaggactggatttcgcctgcttttgggtgctggtggtcgtgggcggagtgctggcttgttattctctgctggtcaccgtggccttcatcatcttttgggtccgactgaagatccaggtccgaaaggccgccatcaccagctacgagaagtctgatggcgtgtacaccggcctgagcaccagaaaccaggaaacctacgagacactgaagcacgagaagcccccccag

SEQ ID NO: 53 - DNA, 6787 bp, synthetic construct
  misc_feature 1..6787: note = artificial sequence
  source 1..6787: mol_type = other DNA
tgtatttagaaaaataaacaaataggggttccgcgcacatttccccgaaaagtgccacctgacgtcgacggatcgggagatctcccgatcccctatggtgcactctcagtacaatctgctctgatgccgcatagttaagccagtatctgctccctgcttgtgtgttggaggtcgctgagtagtgcgcgagcaaaatttaagctacaacaaggcaaggcttgaccgacaattgcatgaagaatctgcttagggttaggcgttttgcgctgcttcgggatccgctgaccaaaagagcaccaaaggcgccctgaccttcagcccctacctgcgctccggtgcccgtcagtgggcagagcgcacatcgcccacagtccccgagaagttggggggaggggtcggcaattgaaccggtgcctagagaaggtggcgcggggtaaactgggaaagtgatgtcgtgtactggctccgcctttttcccgagggtgggggagaaccgtatataagtgcagtagtcgccgtgaacgttctttttcgcaacgggtttgccgccagaacacaggtaagtgccgtgtgtggttcccgcgggcctggcctctttacgggttatggcccttgcgtgccttgaattacttccacctggctgcagtacgtgattcttgatcccgagcttcgggttggaagtgggtgggagagttcgaggccttgcgcttaaggagccccttcgcctcgtgcttgagttgaggcctggcctgggcgctggggccgccgcgtgcgaatctggtggcaccttcgcgcctgtctcgctgctttcgataagtctctagccatttaaaatttttgatgacctgctgcgacgctttttttctggcaagatagtcttgtaaatgcgggccaagatctgcacactggtatttcggtttttggggccgcgggcggcgacggggcccgtgcgtcccagcgcacatgttcggcgaggcggggcctgcgagcgcggccaccgagaatcggacgggggtagtctcaagctggccggcctgctctggtgcctggcctcgcgccgccgtgtatcgccccgccctgggcggcaaggctggcccggtcggcaccagttgcgtgagcggaaagatggccgcttcccggccctgctgcagggagctcaaaatggaggacgcggcgctcgggagagcgggcgggtgagtcacccacacaaaggaaaagggcctttccgtcctcagccgtcgcttcatgtgactccacggagtaccgggcgccgtccaggcacctcgattagttctcgagcttttggagtacgtcgtctttaggttggggggaggggttttatgcgatggagtttccccacactgagtgggtggagactgaagttaggccagcttggcacttgatgtaattctccttggaatttgccctttttgagtttggatcttggttcattctcaagcctcagacagtggttcaaagtttttttcttccatttcaggtgtcgtgataatacgactcactatagggagacccaagctggaattcgccaccatggactggatctggcggattctgtttctcgtgggagctgccacaggcgctcattctgctcagcctgccgatgttgtaatgacgcagtcacccctgtcactcccggtcacacccggagaaccagcgtcaattagctgccgatctagccaaagtttgcttcattccaatggttacaattatctcgactggtacttgcagaaacccggccaatcccctcagctgctcatctaccttgggtctaatagggcatctggggttcccgataggttctctggctccgggagcggcaccgactttacgttgaaaatctctagggttgaggcggaagacgtaggcgtttactattgcatgcaggggacccactggccgctgaccttcggccagggcaccaaggttgaaataaaaggcggcggaggaagcggaggcggaggatctgggggcggaggctctggcggagggggatctcaggtacagctccaggaatcaggacccggtttggttaagccctccgggaccctttccctcacgtgtgcagtctcaggtgggtcaattagttcttccaattggtggtcttgggtgcggcaaccacctggtaaaggtctcgagtggataggggaaatttatcatagtggctccaccaattataacccctcactcaagtccagggttacgatatctgtggacaaaagtaaaaaccaattctccctcaaacttagtagtgtaacagcggcagacaccgcggtgtactactgcgcacggtggacaggccgaactgatgcctttgacatttggggacagggaactatggtgactgtgtcatccgcggccgcgctgagcaacagcatcatgtacttcagccacttcgtgcctgtgttcctgcctgccaagcctacaacaacaccagcccctagacctccaacccctgcccctacaattgcctctcagcctctgtctctgaggcccgaagcttgtagacctgctgctggcggagctgtgcacaccagaggactggatttcgcctgcttttgggtgctggtggtcgtgggcggagtgctggcttgttattctctgctggtcaccgtggccttcatcatcttttgggtccgactgaagatccaggtccgaaaggccgccatcaccagctacgagaagtctgatggcgtgtacaccggcctgagcaccagaaaccaggaaacctacgagacactgaagcacgagaagcccccccagggatctggagctactaacttcagcctgctgaagcaggctggagacgtggaggagaaccctggacctatgtggcagctgctgctgcctacagctctcctgctgctggtgtccgccggcatgagaaccgaggatctgcctaaggccgtggtgttcctggaaccccagtggtacagagtgctggaaaaggacagcgtgaccctgaagtgccagggcgcctacagccccgaggacaatagcacccagtggttccacaacgagagcctgatcagcagccaggccagcagctacttcatcgacgccgccaccgtggacgacagcggcgagtatagatgccagaccaacctgagcaccctgagcgaccccgtgcagctggaagtgcacatcggatggctgctgctgcaggcccccagatgggtgttcaaagaagaggaccccatccacctgagatgccactcttggaagaacaccgccctgcacaaagtgacctacctgcagaacggcaagggcagaaagtacttccaccacaacagcgacttctacatccccaaggccaccctgaaggactccggctcctacttctgcagaggcctcgtgggcagcaagaacgtgtccagcgagacagtgaacatcaccatcacccagggcctggccgtgtctaccatcagcagctttttcccacccggctaccaggtgtccttctgcctcgtgatggtgctgctgttcgccgtggacaccggcctgtacttcagcgtgaaaacaaacatcagaagcagcacccgggactggaaggaccacaagttcaagtggcggaaggacccccaggacaagtgaaattccgcccctctcccccccccccctctccctcccccccccctaacgttactggccgaagccgcttggaataaggccggtgtgcgtttgtctatatgttattttccaccatattgccgtcttttggcaatgtgagggcccggaaacctggccctgtcttcttgacgagcattcctaggggtctttcccctctcgccaaaggaatgcaaggtctgttgaatgtcgtgaaggaagcagttcctctggaagcttcttgaagacaaacaacgtctgtagcgaccctttgcaggcagcggaaccccccacctggcgacaggtgcctctgcggccaaaagccacgtgtataagatacacctgcaaaggcggcacaaccccagtgccacgttgtgagttggatagttgtggaaagagtcaaatggctctcctcaagcgtattcaacaaggggctgaaggatgcccagaaggtaccccattgtatgggatctgatctggggcctcggtgcacatgctttacatgtgtttagtcgaggttaaaaaaacgtctaggccccccgaaccacggggacgtggttttcctttgaaaaacacgataaccgccaccatgtaccggatgcagctgctgagctgtatcgccctgtctctggccctcgtgaccaacagcgcccctaccagcagcagcaccaagaaaacccagctgcagctggaacatctgctgctggacctgcagatgatcctgaacggcatcaacaactacaagaaccccaagctgacccggatgctgaccttcaagttctacatgcccaagaaggccaccgaactgaaacatctgcagtgcctggaagaggaactgaagcccctggaagaagtgctgaacctggcccagagcaagaacttccacctgaggcccagggacctgatcagcaacatcaacgtgatcgtgctggaactgaaaggcagcgagacaaccttcatgtgcgagtacgccgacgagacagctaccatcgtggaatttctgaaccggtggatcaccttctgccagagcatcatcagcaccctgaccggctccgagaaggacgagctgtgagcggccgcccgctgatcagcctcgaacgagatttcgattccaccgccgccttctatgaaaggttgggcttcggaatcgttttccgggacgccggctggatgatcctccagcgcggggatctcatgctggagttcttcgcccaccccaacttgtttattgcagcttataatggttacaaataaagcaatagcatcacaaatttcacaaataaagcatttttttcactgcattctagttgtggtttgtccaaactcatcaatgtatcttatcatgtctgtgcggtgggctctatggcttctgaggcggaaagaaccagctggggctctagggggtatccccggatcctgagcaaaaggccagcaaaaggccaggaaccgtaaaaaggccgcgttgctggcgtttttccataggctccgcccccctgacgagcatcacaaaaatcgacgctcaagtcagaggtggcgaaacccgacaggactataaagataccaggcgtttccccctggaagctccctcgtgcgctctcctgttccgaccctgccgcttaccggatacctgtccgcctttctcccttcgggaagcgtggcgctttctcatagctcacgctgtaggtatctcagttcggtgtaggtcgttcgctccaagctgggctgtgtgcacgaaccccccgttcagcccgaccgctgcgccttatccggtaactatcgtcttgagtccaacccggtaagacacgacttatcgccactggcagcagccactggtaacaggattagcagagcgaggtatgtaggcggtgctacagagttcttgaagtggtggcctaactacggctacactagaagaacagtatttggtatctgcgctctgctgaagccagttaccttcggaaaaagagttggtagctcttgatccggcaaacaaaccaccgctggtagcggtggtttttttgtttgcaagcagcagattacgcgcagaaaaaaaggatctcaagaagatcctttgatcttttctacggggtctgacgctcagtggaacgaaaactcacgttaagggattttggtcatgagattatcaaaaaggatcttcacctagatccttttaaattaaaaatgaagttttaaatcaatctaaagtatatatgagtaaacttggtctgacagttaccaatgcttaatcagtgaggcacctatctcagcgatctgtctatttcgttcatccatagttgcctgactccccgtcgtgtagataactacgatacgggagggcttaccatctggccccagtgctgcaatgataccgcgagaaccacgctcaccggctccagatttatcagcaataaaccagccagccggaagggccgagcgcagaagtggtcctgcaactttatccgcctccatccagtctattaattgttgccgggaagctagagtaagtagttcgccagttaatagtttgcgcaacgttgttgccattgctacaggcatcgtggtgtcacgctcgtcgtttggtatggcttcattcagctccggttcccaacgatcaaggcgagttacatgatcccccatgttgtgcaaaaaagcggttagctccttcggtcctccgatcgttgtcagaagtaagttggccgcagtgttatcactcatggttatggcagcactgcataattctcttactgtcatgccatccgtaagatgcttttctgtgactggtgagtactcaaccaagtcattctgagaatagtgtatgcggcgaccgagttgctcttgcccggcgtcaatacgggataataccgcgccacatagcagaactttaaaagtgctcatcattggaaaacgttcttcggggcgaaaactctcaaggatcttaccgctgttgagatccagttcgatgtaacccactcgtgcacccaactgatcttcagcatcttttactttcaccagcgtttctgggtgagcaaaaacaggaaggcaaaatgccgcaaaaaagggaataagggcgacacggaaatgttgaatactcatactcttcctttttcaatattattgaagcatttatcagggttattgtctcatgagcggatacatatttgaa